European Patent Application EP 4 700 044 A1, published February 25, 2026. Title: PROTEIN ANALOGUE AND USE THEREOF. Applicant: SHANGHAI DUOMIRUI BIOTECHNOLOGY CO., LTD. The sequence listing filed with the application follows.

SEQUENCE LISTING (17 sequences)

SEQ ID NO: 1 - protein, 181 aa, synthetic construct
HPIPDSSPLLQFGGQVRQRYLYTDDAQQTEAHLEIREDGTVGGAADQSPESLLQLKALKPGVIQILGVKTSRFLCQRPDGALYGSLHFDPEACSFRELLLEDGYNVYQSEAHGLPLHLPGNKSPHRDPAPRGPARFLPLPGLPPALPEPPGILAPQPPDVGSSDPLSMVGPSQGRSPSYAS

SEQ ID NO: 2 - protein, 181 aa, synthetic construct
HPIPDSSPLLQFGGQVRQRYLYTDDAQQTEAHLEIREDGTVGGAADQSPESLLQLKALKPGVIQILGVKTSRFLCQRPDGALYGSLHFDPEACSFRERLLEDGYNVYQSEAHGLPLHLPGNKSPHRDPAPRGPARFLPLPGLPPAPPEPPGILAPQPPDVGSSDPLSMVGGSQGRSPSYES

SEQ ID NO: 3 - protein, 288 aa, synthetic construct
MAHHHHHHSSSDSEVNQEAKPEVKPEVKPETHINLKVSDGSSEIFFKIKKTTPLRRLMEAFAKRQGKEMDSLRFLYDGIRIQADQTPEDLDMEDNDIIEAHREQIGGHPIPDSSPLLQFGGQVRQRYLYTDDAQQTEAHLEIREDGTVGGAADQSPESLLQLKALKPGVIQILGVKTSRFLCQRPDGALYGSLHFDPEACSFRERLLEDGYNVYQSEAHGLPLHLPGNKSPHRDPAPRGPARFLPLPGLPPAPPEPPGILAPQPPDVGSSDPLSMVGGSQGRSPSYES

SEQ ID NO: 4 - protein, 181 aa, synthetic construct
HPIPDSSPLLQFGGQVRQRYLYTDDAQCTEAHLEIREDGTVGGAADQSPESLLQLKALKPGVIQILGVKTSRFLCQRPDGALYGSLHFDPEACSFRERLLEDGYNVYQSEAHGLPLHLPGNKSPHRDPAPRGPARFLPLPGLPPAPPEPPGILAPQPPDVGSSDPLSMVGGSQGRSPSYES

SEQ ID NO: 5 - protein, 181 aa, synthetic construct
HPIPDSSPLLQFGGQVRQRYLYTDDAQQTCAHLEIREDGTVGGAADQSPESLLQLKALKPGVIQILGVKTSRFLCQRPDGALYGSLHFDPEACSFRERLLEDGYNVYQSEAHGLPLHLPGNKSPHRDPAPRGPARFLPLPGLPPAPPEPPGILAPQPPDVGSSDPLSMVGGSQGRSPSYES

SEQ ID NO: 6 - protein, 181 aa, synthetic construct
HPIPDSSPLLQFGGQVRQRYLYTDDAQQTEAHLEIRECGTVGGAADQSPESLLQLKALKPGVIQILGVKTSRFLCQRPDGALYGSLHFDPEACSFRERLLEDGYNVYQSEAHGLPLHLPGNKSPHRDPAPRGPARFLPLPGLPPAPPEPPGILAPQPPDVGSSDPLSMVGGSQGRSPSYES

SEQ ID NO: 7 - protein, 181 aa, synthetic construct
HPIPDSSPLLQFGGQVRQRYLYTDDAQQTEAHLEIREDGTVGGAACQSPESLLQLKALKPGVIQILGVKTSRFLCQRPDGALYGSLHFDPEACSFRERLLEDGYNVYQSEAHGLPLHLPGNKSPHRDPAPRGPARFLPLPGLPPAPPEPPGILAPQPPDVGSSDPLSMVGGSQGRSPSYES

SEQ ID NO: 8 - protein, 181 aa, synthetic construct
HPIPDSSPLLQFGGQVRQRYLYTDDAQQTEAHLEIREDGTVGGAADQSPESLLQLKALKPGVIQILGVKTSRFLCQRPDGALYGSLHFDPEACSFRERLLEDGYNVYQSEAHGLPLHLPGNCSPHRDPAPRGPARFLPLPGLPPAPPEPPGILAPQPPDVGSSDPLSMVGGSQGRSPSYES

SEQ ID NO: 9 - protein, 181 aa, synthetic construct
HPIPDSSPLLQFGGQVRQRYLYTDDAQQTEAHLEIREDGTVGGAADQSPESLLQLKALKPGVIQILGVKTSRFLCQRPDGALYGSLHFDPEACSFRERLLEDGYNVYQSEAHGLPLHLPGNKSPCRDPAPRGPARFLPLPGLPPAPPEPPGILAPQPPDVGSSDPLSMVGGSQGRSPSYES

SEQ ID NO: 10 - protein, 232 aa, synthetic construct
SPCASPAAPAPASPAAPAPSAPAAASAAAPAAASAAASAPSAASAAASPAAHPIPDSSPLLQFGGQVRQRYLYTDDAQQTEAHLEIREDGTVGGAADQSPESLLQLKALKPGVIQILGVKTSRFLCQRPDGALYGSLHFDPEACSFRERLLEDGYNVYQSEAHGLPLHLPGNKSPHRDPAPRGPARFLPLPGLPPAPPEPPGILAPQPPDVGSSDPLSMVGGSQGRSPSYES

SEQ ID NO: 11 - protein, 50 aa, synthetic construct
SPASPAAPAPASPAAPAPSAPAAASAAAPAAASAAASAPSAASAAASPAA

SEQ ID NO: 12 - protein, 51 aa, synthetic construct
SPCASPAAPAPASPAAPAPSAPAAASAAAPAAASAAASAPSAASAAASPAA

SEQ ID NO: 13 - protein, 197 aa, synthetic construct
SPCASPAAPAPASPAAHPIPDSSPLLQFGGQVRQRYLYTDDAQQTEAHLEIREDGTVGGAADQSPESLLQLKALKPGVIQILGVKTSRFLCQRPDGALYGSLHFDPEACSFRERLLEDGYNVYQSEAHGLPLHLPGNKSPHRDPAPRGPARFLPLPGLPPAPPEPPGILAPQPPDVGSSDPLSMVGGSQGRSPSYES

SEQ ID NO: 14 - protein, 212 aa, synthetic construct
SPCASPAAPAPASPAAPAPSAPAAASAAAPAHPIPDSSPLLQFGGQVRQRYLYTDDAQQTEAHLEIREDGTVGGAADQSPESLLQLKALKPGVIQILGVKTSRFLCQRPDGALYGSLHFDPEACSFRERLLEDGYNVYQSEAHGLPLHLPGNKSPHRDPAPRGPARFLPLPGLPPAPPEPPGILAPQPPDVGSSDPLSMVGGSQGRSPSYES

SEQ ID NO: 15 - protein, 232 aa, synthetic construct; identical to SEQ ID NO: 10

SEQ ID NO: 16 - protein, 282 aa, synthetic construct
SPCASPAAPAPASPAAPAPSAPAAASAAAPAAASAAASAPSAASAAASPAAPSAPPAAASPAAPSAPPAAASPAAPAPASPAASAPSAPAAASPAAPAPASHPIPDSSPLLQFGGQVRQRYLYTDDAQQTEAHLEIREDGTVGGAADQSPESLLQLKALKPGVIQILGVKTSRFLCQRPDGALYGSLHFDPEACSFRERLLEDGYNVYQSEAHGLPLHLPGNKSPHRDPAPRGPARFLPLPGLPPAPPEPPGILAPQPPDVGSSDPLSMVGGSQGRSPSYES

SEQ ID NO: 17 - protein, 382 aa, synthetic construct
SPCASPAAPAPASPAAPAPSAPAAASAAAPAAASAAASAPSAASAAASPAAPSAPPAAASPAAPSAPPAAASPAAPAPASPAASAPSAPAAASPAAPAPASPAAPAPSAPAAASAAAPAAASAAASAPSASAAASAAAPAAASAAASAPSAASSAASPAAPSAPPAAASPAAPSAPPAAASPAAPAPASPAAPAPSAPAAAHPIPDSSPLLQFGGQVRQRYLYTDDAQQTEAHLEIREDGTVGGAADQSPESLLQLKALKPGVIQILGVKTSRFLCQRPDGALYGSLHFDPEACSFRERLLEDGYNVYQSEAHGLPLHLPGNKSPHRDPAPRGPARFLPLPGLPPAPPEPPGILAPQPPDVGSSDPLSMVGGSQGRSPSYES